European Patent Application EP 4 772 609 A1, published July 8, 2026. Title: Novel Lactic Acid Bacteria and Use Thereof. Applicant: 동화약품주식회사. The sequence listing filed with the application follows.

SEQUENCE LISTING (30 sequences)

SEQ ID NO: 1 - DNA, 779 bp, Bifidobacterium bifidum
  source 1..779: mol_type = other DNA
tacgacttagtcccaatcacgagcctcaccttagacggctccatcccacaaggggttaggccaccggcttcgggtgctgcccactttcatgacttgacgggcggtgtgtacaaggcccgggaacgcattcaccgcggcgttgctgatccgcgattactagcgactccgccttcacggagccggttgcaggctccgatccgaactgagaccggttttcagggatccgctccatgtcgccatgtcgcatcccgctgtaccggccattgtagcatgcgtgaagccctggacgtaaggggcatgatgatctgacgtcatccccaccttcctccgagttaaccccggcggtcccccgtgagttcccaccataacgtgctggcaacacggggcgagggttgcgctcgttgcgggacttaacccaacatctcacgacacgagctgacgacgaccatgcaccacctgtgaacccgccccgaagggaaacgccatctctggcgtcgtcgggaacatgtcaagcccaggtaaggttcttcgcgttgcatcgaattaatccgcatgctccgccgcttgtgcgggcccccgtcaatttctttgagttttagccttgcggccgtactccccaggcgggacgcttaacgcgttagctccgacacggaacacgtggaacgtgccccacatccagcgtccaccgtttacggcgtggactaccagggtatctaatcctgttcgctccccacgctttcgctcctcagcgtcagtgacggcccagagacctgccttcg

SEQ ID NO: 2 - DNA, 779 bp, Lactobacillus paracasei
  source 1..779: mol_type = other DNA
atggctcaggatgaacgctggcggcgtgcctaatacatgcaagtcgaacgagttctcgttgatgatcggtgcttgcaccgagattcaacatggaacgagtggcggacgggtgagtaacacgtgggtaacctgcccttaagtgggggataacatttggaaacagatgctaataccgcatagatccaagaaccgcatggttcttggctgaaagatggcgtaagctatcgcttttggatggacccgcggcgtattagctagttggtgaggtaatggctcaccaaggcgatgatacgtagccgaactgagaggttgatggccacattgggactgagacacggcccaaactcctacgggaggcagcagtagggaatcttccacaatggacgcaagtctgatggagcaacgccgcgtgagtgaagaaggctttcgggtcgtaaaactctgttgttggagaagaatggtcggcagagtaactgttgtcggcgtgacggtatccaaccagaaagccacggctaactacgtgccagcagccgcggtaatacgtaggtggcaagcgttatccggatttattgggcgtaaagcgagcgcaggcggttttttaagtctgatgtgaaagccctcggcttaaccgaggaagcgcatcggaaactgggaaacttgagtgcagaagaggacagtggaactccatgtgtagcggtgaaatgcgtagatatatggaagaacaccagtggcgaaggcggctgtctggtctgtaactgacgctgaggctcgaaagcatg

SEQ ID NO: 3 - DNA, 27 bp, synthetic construct
  source 1..27: mol_type = other DNA
agccaagacaatagagatgcctacttc

SEQ ID NO: 4 - DNA, 25 bp, synthetic construct
  source 1..25: mol_type = other DNA
ggccttgaactcatagagatccaac

SEQ ID NO: 5 - DNA, 20 bp, synthetic construct
  source 1..20: mol_type = other DNA
aaggaagatgaacgctgtca

SEQ ID NO: 6 - DNA, 23 bp, synthetic construct
  source 1..23: mol_type = other DNA
attgcctcccagataaagtatgt

SEQ ID NO: 7 - DNA, 20 bp, synthetic construct
  source 1..20: mol_type = other DNA
gattatggctcagggtccaa

SEQ ID NO: 8 - DNA, 20 bp, synthetic construct
  source 1..20: mol_type = other DNA
gctccagtgaattcggaaag

SEQ ID NO: 9 - DNA, 23 bp, synthetic construct
  source 1..23: mol_type = other DNA
tagtccttcctaccccaatttcc

SEQ ID NO: 10 - DNA, 21 bp, synthetic construct
  source 1..21: mol_type = other DNA
ttggtccttagccactccttc

SEQ ID NO: 11 - DNA, 20 bp, synthetic construct
  source 1..20: mol_type = other DNA
acaagctgcgggtgaagagc

SEQ ID NO: 12 - DNA, 20 bp, synthetic construct
  source 1..20: mol_type = other DNA
caggacagtgacaaagaacg

SEQ ID NO: 13 - DNA, 23 bp, synthetic construct
  source 1..23: mol_type = other DNA
gcaagacggtgactgtgaaggag

SEQ ID NO: 14 - DNA, 22 bp, synthetic construct
  source 1..22: mol_type = other DNA
ggttgacggtgacgcagaagag

SEQ ID NO: 15 - DNA, 20 bp, synthetic construct
  source 1..20: mol_type = other DNA
aagcgaagagtaaggctgtc

SEQ ID NO: 16 - DNA, 20 bp, synthetic construct
  source 1..20: mol_type = other DNA
gtgattgcttgcaaaggaac

SEQ ID NO: 17 - DNA, 20 bp, synthetic construct
  source 1..20: mol_type = other DNA
caccgtctggatgaggctga

SEQ ID NO: 18 - DNA, 22 bp, synthetic construct
  source 1..22: mol_type = other DNA
tgtttgcgcagacccttgatag

SEQ ID NO: 19 - DNA, 22 bp, synthetic construct
  source 1..22: mol_type = other DNA
gattgacgtggagaggtctaac

SEQ ID NO: 20 - DNA, 22 bp, synthetic construct
  source 1..22: mol_type = other DNA
cctgagtttcctcgtacttctg

SEQ ID NO: 21 - DNA, 22 bp, synthetic construct
  source 1..22: mol_type = other DNA
ggctgcctaaagtggagatcct

SEQ ID NO: 22 - DNA, 19 bp, synthetic construct
  source 1..19: mol_type = other DNA
aggcctgtaggcgctcaat

SEQ ID NO: 23 - DNA, 26 bp, synthetic construct
  source 1..26: mol_type = other DNA
tgatgtgaatgacttggatacagaca

SEQ ID NO: 24 - DNA, 26 bp, synthetic construct
  source 1..26: mol_type = other DNA
gctcattgttgtactggttggatatg

SEQ ID NO: 25 - DNA, 22 bp, synthetic construct
  source 1..22: mol_type = other DNA
agggaacctttgcctcatctac

SEQ ID NO: 26 - DNA, 23 bp, synthetic construct
  source 1..23: mol_type = other DNA
ggtggcaactctgataaatgaac

SEQ ID NO: 27 - DNA, 22 bp, synthetic construct
  source 1..22: mol_type = other DNA
ttttatctgcatctgagtttaa

SEQ ID NO: 28 - DNA, 21 bp, synthetic construct
  source 1..21: mol_type = other DNA
ccacttcatcttaccatttat

SEQ ID NO: 29 - DNA, 20 bp, synthetic construct
  source 1..20: mol_type = other DNA
ccatcctgcgtctggacctg

SEQ ID NO: 30 - DNA, 20 bp, synthetic construct
  source 1..20: mol_type = other DNA
ctcgtcatactcctgcttgc